European Patent Application EP 4 729 471 A2, published April 22, 2026. Title: Novel Ligand Assays. Applicant: InsituGen Limited. Application EP. The sequence listing filed with the application follows.

SEQUENCE LISTING (80 sequences)

SEQ ID NO: 1 - DNA, 18 bp, synthetic construct
  misc_feature 1..18: note = T7 RNA polymerase promoter/initiator sequence
  source 1..18: mol_type = other DNA
taatacgactcactatag

SEQ ID NO: 2 - DNA, 18 bp, synthetic construct
  misc_feature 1..18: note = T3 RNA polymerase promoter/initiator sequence
  source 1..18: mol_type = other DNA
aattaaccctcactaaag

SEQ ID NO: 3 - DNA, 18 bp, synthetic construct
  misc_feature 1..18: note = SP6 RNA polymerase promoter/initiator sequence
  source 1..18: mol_type = other DNA
atttaggtgacactatag

SEQ ID NO: 4 - DNA, 15 bp, synthetic construct
  misc_feature 1..15: note = Androgen Response Element 1 - Sense Strand
  source 1..15: mol_type = other DNA
agaacannntgttct

SEQ ID NO: 5 - DNA, 15 bp, synthetic construct
  misc_feature 1..15: note = Androgen Response Element 1 - Antisense Strand
  source 1..15: mol_type = other DNA
agaacannntgttct

SEQ ID NO: 6 - DNA, 15 bp, synthetic construct
  misc_feature 1..15: note = Androgen Response Element 2 - Sense Strand
  source 1..15: mol_type = other DNA
ggtacannntgttct

SEQ ID NO: 7 - DNA, 15 bp, synthetic construct
  misc_feature 1..15: note = Androgen Response Element 2 - Antisense Strand
  source 1..15: mol_type = other DNA
agaacannntgtacc

SEQ ID NO: 8 - DNA, 15 bp, synthetic construct
  misc_feature 1..15: note = Estrogen Response Element - Sense Strand
  source 1..15: mol_type = other DNA
aggtcannntgacct

SEQ ID NO: 9 - DNA, 15 bp, synthetic construct
  misc_feature 1..15: note = Estrogen Response Element - Sense Strand
  source 1..15: mol_type = other DNA
aggtcannntgacct

SEQ ID NO: 10 - DNA, 15 bp, synthetic construct
  misc_feature 1..15: note = Progesterone Response Element - Sense Strand
  source 1..15: mol_type = other DNA
ggtacaaactgttct

SEQ ID NO: 11 - DNA, 15 bp, synthetic construct
  misc_feature 1..15: note = Progesterone Response Element - Antisense Strand
  source 1..15: mol_type = other DNA
agaacagtttgtacc

SEQ ID NO: 12 - DNA, 15 bp, synthetic construct
  misc_feature 1..15: note = Glucocorticoid/Mineralocorticoid Response Element - Sense Strand
  source 1..15: mol_type = other DNA
agaacanaatgttct

SEQ ID NO: 13 - DNA, 15 bp, synthetic construct
  misc_feature 1..15: note = Glucocorticoid/Mineralocorticoid Response Element - Antisense Strand
  source 1..15: mol_type = other DNA
agaacattntgttct

SEQ ID NO: 14 - DNA, 146 bp, synthetic construct
  misc_feature 1..146: note = T7i-ARE-F30MangoII
  source 1..146: mol_type = other DNA
taatacgactcactatagactctggaggaatggagaacagcctgttctccattgccatgtgtatgtgggtacgaaggagaggagaggaagaggagagtacccacatactctgatgatccttcgggatcattcatggcaatctagga

SEQ ID NO: 15 - DNA, 142 bp, synthetic construct
  misc_feature 1..142: note = T7i-ERE-F30MangoII
  source 1..142: mol_type = other DNA
taatacgactcactatagactctggaggaacaggtcagcatgacctgttgccatgtgtatgtgggtacgaaggagaggagaggaagaggagagtacccacatactctgatgatccttcgggatcattcatggcaatctagga

SEQ ID NO: 16 - DNA, 140 bp, synthetic construct
  misc_feature 1..140: note = T7i-PRE-F30MangoII
  source 1..140: mol_type = other DNA
taatacgactcactatagactctggaggaaggtacaaactgttctttgccatgtgtatgtgggtacgaaggagaggagaggaagaggagagtacccacatactctgatgatccttcgggatcattcatggcaatctagga

SEQ ID NO: 17 - DNA, 140 bp, synthetic construct
  misc_feature 1..140: note = T7i-MRE-F30MangoII
  source 1..140: mol_type = other DNA
taatacgactcactatagactctggaggaatgtacaggatgttctttgccatgtgtatgtgggtacgaaggagaggagaggaagaggagagtacccacatactctgatgatccttcgggatcattcatggcaatctagga

SEQ ID NO: 18 - DNA, 140 bp, synthetic construct; identical to SEQ ID NO: 17
  misc_feature 1..140: note = T7i-GRE-F30MangoII
  source 1..140: mol_type = other DNA

SEQ ID NO: 19 - DNA, 81 bp, synthetic construct
  misc_feature 1..81: note = T7i-ARE-MangoII
  source 1..81: mol_type = other DNA
taatacgactcactatagactctggaggaatggagaacagcctgttctccatacgaaggagaggagaggaagaggagagta

SEQ ID NO: 20 - DNA, 77 bp, synthetic construct
  misc_feature 1..77: note = T7i-ERE-MangoII
  source 1..77: mol_type = other DNA
taatacgactcactatagactctggaggaacaggtcagcatgacctgtacgaaggagaggagaggaagaggagagta

SEQ ID NO: 21 - DNA, 75 bp, synthetic construct
  misc_feature 1..75: note = T7i-PRE-MangoII
  source 1..75: mol_type = other DNA
taatacgactcactatagactctggaggaaggtacaaactgttcttacgaaggagaggagaggaagaggagagta

SEQ ID NO: 22 - DNA, 75 bp, synthetic construct
  misc_feature 1..75: note = T7i-MRE-MangoII
  source 1..75: mol_type = other DNA
taatacgactcactatagactctggaggaatgtacaggatgttcttacgaaggagaggagaggaagaggagagta

SEQ ID NO: 23 - DNA, 75 bp, synthetic construct; identical to SEQ ID NO: 22
  misc_feature 1..75: note = T7i-GRE-MangoII
  source 1..75: mol_type = other DNA

SEQ ID NO: 24 - DNA, 120 bp, synthetic construct
  misc_feature 1..120: note = T7i-ARE-iSpinach
  source 1..120: mol_type = other DNA
taatacgactcactatagactctggaggaatggagaacagcctgttctccaaggagtacggtgagggtcgggtccagtaggtacgcctactgttgagtagagtgtgggctccgtactccc

SEQ ID NO: 25 - DNA, 116 bp, synthetic construct
  misc_feature 1..116: note = T7i-ERE-iSpinach
  source 1..116: mol_type = other DNA
taatacgactcactatagactctggaggaacaggtcagcatgacctgaggagtacggtgagggtcgggtccagtaggtacgcctactgttgagtagagtgtgggctccgtactccc

SEQ ID NO: 26 - DNA, 114 bp, synthetic construct
  misc_feature 1..114: note = T7i-PRE-iSpinach
  source 1..114: mol_type = other DNA
taatacgactcactatagactctggaggaaggtacaaactgttctaggagtacggtgagggtcgggtccagtaggtacgcctactgttgagtagagtgtgggctccgtactccc

SEQ ID NO: 27 - DNA, 114 bp, synthetic construct
  misc_feature 1..114: note = T7i-MRE-iSpinach
  source 1..114: mol_type = other DNA
taatacgactcactatagactctggaggaatgtacaggatgttctaggagtacggtgagggtcgggtccagtaggtacgcctactgttgagtagagtgtgggctccgtactccc

SEQ ID NO: 28 - DNA, 114 bp, synthetic construct; identical to SEQ ID NO: 27
  misc_feature 1..114: note = T7i-GRE-iSpinach
  source 1..114: mol_type = other DNA

SEQ ID NO: 29 - DNA, 190 bp, synthetic construct
  misc_feature 1..190: note = T7i-ARE-F30iSpinach
  source 1..190: mol_type = other DNA
taatacgactcactatagactctggaggaatggagaacagcctgttctccattgccatgtgtatgtgggaggagtacggtgagggtcgggtccagtaggtacgcctactgttgagtagagtgtgggctccgtactccccccacatactctgatgatccttcgggatcattcatggcaatctagatctaga

SEQ ID NO: 30 - DNA, 186 bp, synthetic construct
  misc_feature 1..186: note = T7i-ERE-F30iSpinach
  source 1..186: mol_type = other DNA
taatacgactcactatagactctggaggaacaggtcagcatgacctgttgccatgtgtatgtgggaggagtacggtgagggtcgggtccagtaggtacgcctactgttgagtagagtgtgggctccgtactccccccacatactctgatgatccttcgggatcattcatggcaatctagatctaga

SEQ ID NO: 31 - DNA, 184 bp, synthetic construct
  misc_feature 1..184: note = T7i-PRE-F30iSpinach
  source 1..184: mol_type = other DNA
taatacgactcactatagactctggaggaaggtacaaactgttctttgccatgtgtatgtgggaggagtacggtgagggtcgggtccagtaggtacgcctactgttgagtagagtgtgggctccgtactccccccacatactctgatgatccttcgggatcattcatggcaatctagatctaga

SEQ ID NO: 32 - DNA, 184 bp, synthetic construct
  misc_feature 1..184: note = T7i-MRE-F30iSpinach
  source 1..184: mol_type = other DNA
taatacgactcactatagactctggaggaatgtacaggatgttctttgccatgtgtatgtgggaggagtacggtgagggtcgggtccagtaggtacgcctactgttgagtagagtgtgggctccgtactccccccacatactctgatgatccttcgggatcattcatggcaatctagatctaga

SEQ ID NO: 33 - DNA, 184 bp, synthetic construct; identical to SEQ ID NO: 32
  misc_feature 1..184: note = T7i-GRE-F30iSpinach
  source 1..184: mol_type = other DNA

SEQ ID NO: 34 - DNA, 81 bp, synthetic construct
  misc_feature 1..81: note = T3i-ARE-MangoII
  source 1..81: mol_type = other DNA
aattaaccctcactaaagactctggaggaatggagaacagcctgttctccatacgaaggagaggagaggaagaggagagta

SEQ ID NO: 35 - DNA, 77 bp, synthetic construct
  misc_feature 1..77: note = T3i-ERE-MangoII
  source 1..77: mol_type = other DNA
aattaaccctcactaaagactctggaggaacaggtcagcatgacctgtacgaaggagaggagaggaagaggagagta

SEQ ID NO: 36 - DNA, 75 bp, synthetic construct
  misc_feature 1..75: note = T3i-PRE-MangoII
  source 1..75: mol_type = other DNA
aattaaccctcactaaagactctggaggaaggtacaaactgttcttacgaaggagaggagaggaagaggagagta

SEQ ID NO: 37 - DNA, 75 bp, synthetic construct
  misc_feature 1..75: note = T3i-MRE-MangoII
  source 1..75: mol_type = other DNA
aattaaccctcactaaagactctggaggaatgtacaggatgttcttacgaaggagaggagaggaagaggagagta

SEQ ID NO: 38 - DNA, 75 bp, synthetic construct; identical to SEQ ID NO: 37
  misc_feature 1..75: note = T3i-GRE-MangoII
  source 1..75: mol_type = other DNA

SEQ ID NO: 39 - DNA, 146 bp, synthetic construct
  misc_feature 1..146: note = T3i-ARE-F30MangoII
  source 1..146: mol_type = other DNA
aattaaccctcactaaagactctggaggaatggagaacagcctgttctccattgccatgtgtatgtgggtacgaaggagaggagaggaagaggagagtacccacatactctgatgatccttcgggatcattcatggcaatctagga

SEQ ID NO: 40 - DNA, 142 bp, synthetic construct
  misc_feature 1..142: note = T3i-ERE-F30MangoII
  source 1..142: mol_type = other DNA
aattaaccctcactaaagactctggaggaacaggtcagcatgacctgttgccatgtgtatgtgggtacgaaggagaggagaggaagaggagagtacccacatactctgatgatccttcgggatcattcatggcaatctagga

SEQ ID NO: 41 - DNA, 140 bp, synthetic construct
  misc_feature 1..140: note = T3i-PRE-F30MangoII
  source 1..140: mol_type = other DNA
aattaaccctcactaaagactctggaggaaggtacaaactgttctttgccatgtgtatgtgggtacgaaggagaggagaggaagaggagagtacccacatactctgatgatccttcgggatcattcatggcaatctagga

SEQ ID NO: 42 - DNA, 140 bp, synthetic construct
  misc_feature 1..140: note = T3i-MRE-F30MangoII
  source 1..140: mol_type = other DNA
aattaaccctcactaaagactctggaggaatgtacaggatgttctttgccatgtgtatgtgggtacgaaggagaggagaggaagaggagagtacccacatactctgatgatccttcgggatcattcatggcaatctagga

SEQ ID NO: 43 - DNA, 140 bp, synthetic construct; identical to SEQ ID NO: 42
  misc_feature 1..140: note = T3i-GRE-F30MangoII
  source 1..140: mol_type = other DNA

SEQ ID NO: 44 - DNA, 120 bp, synthetic construct
  misc_feature 1..120: note = T3i-ARE-iSpinach
  source 1..120: mol_type = other DNA
aattaaccctcactaaagactctggaggaatggagaacagcctgttctccaaggagtacggtgagggtcgggtccagtaggtacgcctactgttgagtagagtgtgggctccgtactccc

SEQ ID NO: 45 - DNA, 116 bp, synthetic construct
  misc_feature 1..116: note = T3i-ERE-iSpinach
  source 1..116: mol_type = other DNA
aattaaccctcactaaagactctggaggaacaggtcagcatgacctgaggagtacggtgagggtcgggtccagtaggtacgcctactgttgagtagagtgtgggctccgtactccc

SEQ ID NO: 46 - DNA, 114 bp, synthetic construct
  misc_feature 1..114: note = T3i-PRE-iSpinach
  source 1..114: mol_type = other DNA
aattaaccctcactaaagactctggaggaaggtacaaactgttctaggagtacggtgagggtcgggtccagtaggtacgcctactgttgagtagagtgtgggctccgtactccc

SEQ ID NO: 47 - DNA, 114 bp, synthetic construct
  misc_feature 1..114: note = T3i-MRE-iSpinach
  source 1..114: mol_type = other DNA
aattaaccctcactaaagactctggaggaatgtacaggatgttctaggagtacggtgagggtcgggtccagtaggtacgcctactgttgagtagagtgtgggctccgtactccc

SEQ ID NO: 48 - DNA, 114 bp, synthetic construct; identical to SEQ ID NO: 47
  misc_feature 1..114: note = T3i-GRE-iSpinach
  source 1..114: mol_type = other DNA

SEQ ID NO: 49 - DNA, 190 bp, synthetic construct
  misc_feature 1..190: note = T3i-ARE-F30iSpinach
  source 1..190: mol_type = other DNA
aattaaccctcactaaagactctggaggaatggagaacagcctgttctccattgccatgtgtatgtgggaggagtacggtgagggtcgggtccagtaggtacgcctactgttgagtagagtgtgggctccgtactccccccacatactctgatgatccttcgggatcattcatggcaatctagatctaga

SEQ ID NO: 50 - DNA, 186 bp, synthetic construct
  misc_feature 1..186: note = T3i-ERE- F30iSpinach
  source 1..186: mol_type = other DNA
aattaaccctcactaaagactctggaggaacaggtcagcatgacctgttgccatgtgtatgtgggaggagtacggtgagggtcgggtccagtaggtacgcctactgttgagtagagtgtgggctccgtactccccccacatactctgatgatccttcgggatcattcatggcaatctagatctaga

SEQ ID NO: 51 - DNA, 184 bp, synthetic construct
  misc_feature 1..184: note = T3i-PRE- F30iSpinach
  source 1..184: mol_type = other DNA
aattaaccctcactaaagactctggaggaaggtacaaactgttctttgccatgtgtatgtgggaggagtacggtgagggtcgggtccagtaggtacgcctactgttgagtagagtgtgggctccgtactccccccacatactctgatgatccttcgggatcattcatggcaatctagatctaga

SEQ ID NO: 52 - DNA, 184 bp, synthetic construct
  misc_feature 1..184: note = T3i-MRE- F30iSpinach
  source 1..184: mol_type = other DNA
aattaaccctcactaaagactctggaggaatgtacaggatgttctttgccatgtgtatgtgggaggagtacggtgagggtcgggtccagtaggtacgcctactgttgagtagagtgtgggctccgtactccccccacatactctgatgatccttcgggatcattcatggcaatctagatctaga

SEQ ID NO: 53 - DNA, 184 bp, synthetic construct; identical to SEQ ID NO: 52
  misc_feature 1..184: note = T3i-GRE- F30iSpinach
  source 1..184: mol_type = other DNA

SEQ ID NO: 54 - DNA, 81 bp, synthetic construct
  misc_feature 1..81: note = SP6i-ARE-MangoII
  source 1..81: mol_type = other DNA
atttaggtgacactatagactctggaggaatggagaacagcctgttctccatacgaaggagaggagaggaagaggagagta

SEQ ID NO: 55 - DNA, 77 bp, synthetic construct
  misc_feature 1..77: note = SP6i-ERE-MangoII
  source 1..77: mol_type = other DNA
atttaggtgacactatagactctggaggaacaggtcagcatgacctgtacgaaggagaggagaggaagaggagagta

SEQ ID NO: 56 - DNA, 75 bp, synthetic construct
  misc_feature 1..75: note = SP6i-PRE-MangoII
  source 1..75: mol_type = other DNA
atttaggtgacactatagactctggaggaaggtacaaactgttcttacgaaggagaggagaggaagaggagagta

SEQ ID NO: 57 - DNA, 75 bp, synthetic construct
  misc_feature 1..75: note = SP6i-MRE-MangoII
  source 1..75: mol_type = other DNA
atttaggtgacactatagactctggaggaatgtacaggatgttcttacgaaggagaggagaggaagaggagagta

SEQ ID NO: 58 - DNA, 75 bp, synthetic construct; identical to SEQ ID NO: 57
  misc_feature 1..75: note = SP6i-GRE-MangoII
  source 1..75: mol_type = other DNA

SEQ ID NO: 59 - DNA, 146 bp, synthetic construct
  misc_feature 1..146: note = SP6i-ARE-F30MangoII
  source 1..146: mol_type = other DNA
atttaggtgacactatagactctggaggaatggagaacagcctgttctccattgccatgtgtatgtgggtacgaaggagaggagaggaagaggagagtacccacatactctgatgatccttcgggatcattcatggcaatctagga

SEQ ID NO: 60 - DNA, 142 bp, synthetic construct
  misc_feature 1..142: note = SP6i-ERE-F30MangoII
  source 1..142: mol_type = other DNA
atttaggtgacactatagactctggaggaacaggtcagcatgacctgttgccatgtgtatgtgggtacgaaggagaggagaggaagaggagagtacccacatactctgatgatccttcgggatcattcatggcaatctagga

SEQ ID NO: 61 - DNA, 140 bp, synthetic construct
  misc_feature 1..140: note = SP6i-PRE-F30MangoII
  source 1..140: mol_type = other DNA
atttaggtgacactatagactctggaggaaggtacaaactgttctttgccatgtgtatgtgggtacgaaggagaggagaggaagaggagagtacccacatactctgatgatccttcgggatcattcatggcaatctagga

SEQ ID NO: 62 - DNA, 140 bp, synthetic construct
  misc_feature 1..140: note = SP6i-MRE-F30MangoII
  source 1..140: mol_type = other DNA
atttaggtgacactatagactctggaggaatgtacaggatgttctttgccatgtgtatgtgggtacgaaggagaggagaggaagaggagagtacccacatactctgatgatccttcgggatcattcatggcaatctagga

SEQ ID NO: 63 - DNA, 140 bp, synthetic construct; identical to SEQ ID NO: 62
  misc_feature 1..140: note = SP6i-GRE-F30MangoII
  source 1..140: mol_type = other DNA

SEQ ID NO: 64 - DNA, 120 bp, synthetic construct
  misc_feature 1..120: note = SP6i-ARE-iSpinach
  source 1..120: mol_type = other DNA
atttaggtgacactatagactctggaggaatggagaacagcctgttctccaaggagtacggtgagggtcgggtccagtaggtacgcctactgttgagtagagtgtgggctccgtactccc

SEQ ID NO: 65 - DNA, 116 bp, synthetic construct
  misc_feature 1..116: note = SP6i-ERE-iSpinach
  source 1..116: mol_type = other DNA
atttaggtgacactatagactctggaggaacaggtcagcatgacctgaggagtacggtgagggtcgggtccagtaggtacgcctactgttgagtagagtgtgggctccgtactccc

SEQ ID NO: 66 - DNA, 114 bp, synthetic construct
  misc_feature 1..114: note = SP6i-PRE-iSpinach
  source 1..114: mol_type = other DNA
atttaggtgacactatagactctggaggaaggtacaaactgttctaggagtacggtgagggtcgggtccagtaggtacgcctactgttgagtagagtgtgggctccgtactccc

SEQ ID NO: 67 - DNA, 114 bp, synthetic construct
  misc_feature 1..114: note = SP6i-MRE-iSpinach
  source 1..114: mol_type = other DNA
atttaggtgacactatagactctggaggaatgtacaggatgttctaggagtacggtgagggtcgggtccagtaggtacgcctactgttgagtagagtgtgggctccgtactccc

SEQ ID NO: 68 - DNA, 114 bp, synthetic construct; identical to SEQ ID NO: 67
  misc_feature 1..114: note = SP6i-GRE-iSpinach
  source 1..114: mol_type = other DNA

SEQ ID NO: 69 - DNA, 190 bp, synthetic construct
  misc_feature 1..190: note = SP6i-ARE-F30iSpinach
  source 1..190: mol_type = other DNA
atttaggtgacactatagactctggaggaatggagaacagcctgttctccattgccatgtgtatgtgggaggagtacggtgagggtcgggtccagtaggtacgcctactgttgagtagagtgtgggctccgtactccccccacatactctgatgatccttcgggatcattcatggcaatctagatctaga

SEQ ID NO: 70 - DNA, 186 bp, synthetic construct
  misc_feature 1..186: note = SP6i-ERE- F30iSpinach
  source 1..186: mol_type = other DNA
atttaggtgacactatagactctggaggaacaggtcagcatgacctgttgccatgtgtatgtgggaggagtacggtgagggtcgggtccagtaggtacgcctactgttgagtagagtgtgggctccgtactccccccacatactctgatgatccttcgggatcattcatggcaatctagatctaga

SEQ ID NO: 71 - DNA, 184 bp, synthetic construct
  misc_feature 1..184: note = SP6i-PRE- F30iSpinach
  source 1..184: mol_type = other DNA
atttaggtgacactatagactctggaggaaggtacaaactgttctttgccatgtgtatgtgggaggagtacggtgagggtcgggtccagtaggtacgcctactgttgagtagagtgtgggctccgtactccccccacatactctgatgatccttcgggatcattcatggcaatctagatctaga

SEQ ID NO: 72 - DNA, 184 bp, synthetic construct
  misc_feature 1..184: note = SP6i-MRE-F30iSpinach
  source 1..184: mol_type = other DNA
atttaggtgacactatagactctggaggaatgtacaggatgttctttgccatgtgtatgtgggaggagtacggtgagggtcgggtccagtaggtacgcctactgttgagtagagtgtgggctccgtactccccccacatactctgatgatccttcgggatcattcatggcaatctagatctaga

SEQ ID NO: 73 - DNA, 184 bp, synthetic construct; identical to SEQ ID NO: 72
  misc_feature 1..184: note = SP6i-GRE-F30iSpinach
  source 1..184: mol_type = other DNA

SEQ ID NO: 74 - DNA, 12 bp, synthetic construct
  misc_feature 1..12: note = Filler Sequence
  source 1..12: mol_type = other DNA
actctggaggaa

SEQ ID NO: 75 - DNA, 67 bp, synthetic construct
  misc_feature 1..67: note = 3xTandem Androgen Response Element
  source 1..67: mol_type = other DNA
aagcttagaacagtttgtaacgagctcgttacaaactgttctagctcgttacaaactgttctaagct

SEQ ID NO: 76 - DNA, 21 bp, synthetic construct
  misc_feature 1..21: note = Primary Androgen Response Element
  source 1..21: mol_type = other DNA
tggagaacagcctgttctcca

SEQ ID NO: 77 - DNA, 95 bp, synthetic construct
  misc_feature 1..95: note = MangoII Aptamer + F30 Scaffold
  source 1..95: mol_type = other DNA
ttgccatgtgtatgtgggtacgaaggagaggagaggaagaggagagtacccacatactctgatgatccttcgggatcattcatggcaatctagga

SEQ ID NO: 78 - DNA, 30 bp, synthetic construct
  misc_feature 1..30: note = MangoII Aptamer
  source 1..30: mol_type = other DNA
tacgaaggagaggagaggaagaggagagta

SEQ ID NO: 79 - DNA, 17 bp, synthetic construct
  misc_feature 1..17: note = Primary Estrogen Response Element
  source 1..17: mol_type = other DNA
caggtcagcatgacctg

SEQ ID NO: 80 - DNA, 331 bp, synthetic construct
  misc_feature 1..331: note = ARE/ERE Multiplexed Assay (Single) Nucleic Acid Molecule
  source 1..331: mol_type = other DNA
taatacgactcactatagactctggaggaatggagaacagcctgttctccattgccatgtgtatgtgggtacgaaggagaggagaggaagaggagagtacccacatactctgatgatccttcgggatcattcatggcaatctaggaaaccccgcggggcctttcgggggtctcgcggggttttttgctctaatacgactcactatagactctggaggaacaggtcagcatgacctgttgccatgtgtatgtgggtacgaaggagaggagaggaagaggagagtacccacatactctgatgatccttcgggatcattcatggcaatctagga